European Patent Application EP 4 810 056 A2, published September 23, 2026. Title: METHODS AND COMBINATIONS FOR TREATING CERVICAL CANCER. Applicant: AstraZeneca AB. Application US. The sequence listing filed with the application follows.

SEQUENCE LISTING (16 sequences)

SEQ ID NO: 1 - protein, 219 aa, synthetic construct
QIVLTQSPATLSLSPGERATLSCSASSKHTNLYWSRHMYWYQQKPGQAPRLLIYLTSNRATGIPARFSGSGSGTDFTLTISSLEPEDFAVYYCQQWSSNPFTFGQGTKLEIKRTVAAPSVFIFPPSDEQLKSGTASVVCLLNNFYPREAKVQWKVDNALQSGNSQESVTEQDSKDSTYSLSSTLTLSKADYEKHKVYACEVTHQGLSSPVTKSFNRGEC

SEQ ID NO: 2 - protein, 452 aa, synthetic construct
EVQLVESGGGLVQPGGSLRLSCAASGFTFSDYGMHWVRQAPGKGLEWVAYISSGSYTIYSADSVKGRFTISRDNAKNSLYLQMNSLRAEDTAVYYCARRAPNSFYEYYFDYWGQGTTVTVSSASTKGPSVFPLAPSSKSTSGGTAALGCLVKDYFPEPVTVSWNSGALTSGVHTFPAVLQSSGLYSLSSVVTVPSSSLGTQTYICNVNHKPSNTKVDKRVEPKSCDKTHTCPPCPAPEFEGGPSVFLFPPKPKDTLMISRTPEVTCVVVDVSHEDPEVKFNWYVDGVEVHNAKTKPREEQYNSTYRVVSVLTVLHQDWLNGKEYKCKVSNKALPASIEKTISKAKGQPREPQVCTLPPSREEMTKNQVSLSCAVKGFYPSDIAVEWESNGQPENNYKTTPPVLDSDGSFFLVSKLTVDKSRWQQGNVFSCSVMHEALHNHYTQKSLSLSPGK

SEQ ID NO: 3 - protein, 213 aa, synthetic construct
DIQMTQSPSSLSASVGDRVTITCRASQSINSYLDWYQQKPGKAPKLLIYAASSLQSGVPSRFSGSGSGTDFTLTISSLQPEDFATYYCQQYYSTPFTFGPGTKVEIKGQPKAAPSVTLFPPCSEELQANKATLVCLISDFYPGAVTVAWKADSSPVKAGVETTTPSKQSNNKYAASSYLSLTPEQWKSHRSYSCQVTHEGSTVEKTVAPTEVS

SEQ ID NO: 4 - protein, 455 aa, synthetic construct
QVQLVESGGGVVQPGRSLRLSCAASGFTFSSYGMHWVRQAPGKGLEWVAVIWYDGSNKYYADSVKGRFTISRDNSKNTLYLQMNSLRAEDTAVYYCARDPRGATLYYYYYGMDVWGQGTTVTVSSASTKGPSVCPLAPSSKSTSGGTAALGCLVKDYFPEPVTVSWNSGALTSGVHTFPAVLQSSGLYSLSSVVTVPSSSLGTQTYICNVNHKPSNTKVDKRVEPKSVDKTHTCPPCPAPEFEGGPSVFLFPPKPKDTLMISRTPEVTCVVVDVSHEDPEVKFNWYVDGVEVHNAKTKPREEQYNSTYRVVSVLTVLHQDWLNGKEYKCKVSNKALPASIEKTISKAKGQPREPQVYTLPPCREEMTKNQVSLWCLVKGFYPSDIAVEWESNGQPENNYKTTPPVLDSDGSFFLYSKLTVDKSRWQQGNVFSCSVMHEALHNHYTQKSLSLSPGK

SEQ ID NO: 5 - protein, 18 aa, synthetic construct
SASSKHTNLYWSRHMYWY

SEQ ID NO: 6 - protein, 6 aa, synthetic construct
TSNRAT

SEQ ID NO: 7 - protein, 7 aa, synthetic construct
QQWSSNP

SEQ ID NO: 8 - protein, 10 aa, synthetic construct
GFTFSDYGMH

SEQ ID NO: 9 - protein, 17 aa, synthetic construct
YISSGSYTIYSADSVKG

SEQ ID NO: 10 - protein, 13 aa, synthetic construct
RAPNSFYEYYFDY

SEQ ID NO: 11 - protein, 11 aa, synthetic construct
RASQSINSYLD

SEQ ID NO: 12 - protein, 7 aa, synthetic construct
AASSLQS

SEQ ID NO: 13 - protein, 7 aa, synthetic construct
QQYYSTP

SEQ ID NO: 14 - protein, 10 aa, synthetic construct
GFTFSSYGMH

SEQ ID NO: 15 - protein, 17 aa, synthetic construct
VIWYDGSNKYYADSVKG

SEQ ID NO: 16 - protein, 16 aa, synthetic construct
DPRGATLYYYYYGMDV